European Patent Application EP 4 488 368 A1, published January 8, 2025. Title: NAD(P)H OXIDASE. Applicant: Annikki GmbH. Application EP. The sequence listing filed with the application follows.

SEQUENCE LISTING (23 sequences)

SEQ ID NO: 1 - protein, 451 aa, Carnobacterium divergens
MKVVVVGCTHAGTAAVKTILNEHPDASVSVYERNDNVSFLSCGIALYVGGVVKDPAGLFYSSPEELASMGAKINMEHNVKNIDNENKVVVIENLKTGETFEESYDKLVMTTGSWPIIPPIDGINSENILLCKNYNQANEIIKESKNAKKIVIVGGGYIGIELVEAFAESGKQVTLVDGLDRILNKYLDAEFTSVLEHDLQERGVTLALNQTVEKFVANESGAVTAVKTPVGEYEADLVILCVGFKPNTDLLKDKVEMLPNGAIVVDEYMRTSDEAIFAAGDSCAVHYNPTGGSAYIPLATNAVRMGALVGKNIVSPTVKYRGTQATSGLYLFGFNIGSTGLTENSAPHFGVEVRSVVVEDNYRPEFMPTTEKVTMKLVYEVGTNRIVGGQIMSKYDVTQSANTLSLCVQNKMTIEDLAYVDFFFQPHFDRPWNYLNILAQAAVEQERKLAK

SEQ ID NO: 2 - DNA, 1356 bp, Carnobacterium divergens
  source 1..1356: mol_type = other DNA
atgaaagtagtagtagtaggctgtacacatgcaggaacagcggcagttaagacgattttaaatgaacatccagatgcatcagtatcagtatatgagcgtaatgacaatgtctcatttctatcttgtgggattgcgttgtatgttggtggagttgtgaaagatcctgcaggtttgttttattcaagtccagaagaacttgcatcaatgggcgcgaaaattaacatggaacacaatgtgaaaaatatagataatgagaataaggtcgtagtaattgagaatttaaaaacaggcgaaacatttgaagaaagctatgataagttggtaatgacaactggatcatggccaattattcctccaattgatggaatcaatagtgaaaatattcttttgtgtaaaaactataaccaagcaaatgaaattattaaagaatcaaaaaatgctaaaaagattgtcattgttggtggtggctatattggaattgaattagttgaggcatttgcagaatctggcaagcaagtgacgctagttgatggattagatcgtattttaaacaaatatttagatgctgaattcacttctgttttagagcatgatttacaagaaagaggcgttacgctagctttaaaccaaaccgtcgagaaatttgttgccaatgaatcaggtgctgtgacagctgtgaaaacaccagttggagaatatgaggctgatttagttattttatgtgttggatttaaaccaaatactgatttgttgaaggataaagtagagatgttgccaaatggtgccatcgtagtggatgaatatatgagaacaagcgatgaagcgatttttgctgctggcgatagttgcgcggttcattataatccaactggaggctctgcgtatattccgttagctacaaatgcagttagaatgggagctttagttgggaaaaatattgtttctccaacagttaaatatcgtggcacgcaagcaacttctggtttatatttatttggttttaatataggttcaaccggattgactgaaaatagcgctcctcattttggcgtagaggttcgttcagtagttgtagaagataattatcgtccagagtttatgccgacaacagagaaagtaacgatgaaattagtttatgaagtaggaacgaatcggattgttggaggtcaaatcatgtcaaaatatgatgtgacacaatctgccaatacgttatctttatgtgttcaaaataaaatgacgattgaggatttggcttatgtagatttcttcttccaacctcactttgatcgtccttggaactatttaaatattttagcgcaagcagctgttgagcaagagcgtaaactagcaaaataa

SEQ ID NO: 3 - protein, 6 aa, synthetic construct
  source 1..6: note = enzyme motif
  VARIANT 6: note = a non-polar amino acid residue
GGGYIX

SEQ ID NO: 4 - protein, 6 aa, synthetic construct
  source 1..6: note = enzyme motif
GGGYIG

SEQ ID NO: 5 - protein, 6 aa, synthetic construct
  source 1..6: note = enzyme motif
GGGYIA

SEQ ID NO: 6 - protein, 14 aa, synthetic construct
  source 1..14: note = enzyme motif
  VARIANT 6: note = a non-polar amino acid residue
  VARIANT 7: note = peptide consisting of 6 to 12 amino acid residues
  VARIANT 8: note = a polar amino acid residue
  VARIANT 9: note = a peptide consisting of 4 to 8 amino acid residues
  VARIANT 10: note = an acidic amino acid residue or a non-polar amino acid residue
  VARIANT 11: note = a polar amino acid residue or a basic amino acid residue
  VARIANT 12: note = a non-polar amino acid residue or a polar amino acid residue
  VARIANT 13: note = a peptide consisting of 2 to 6 amino acid residues
  VARIANT 14: note = a polar amino acid residue or a basic amino acid residue
GGGYIXXXXXXXXX

SEQ ID NO: 7 - protein, 14 aa, synthetic construct
  source 1..14: note = enzyme motif
  VARIANT 7: note = a peptide consisting of 6 to 12 amino acid residues
  VARIANT 8: note = a polar amino acid residue
  VARIANT 9: note = a peptide consisting of 4 to 8 amino acid residues
  VARIANT 10: note = an acidic amino acid residue or a non-polar amino acid residue
  VARIANT 11: note = a polar amino acid residue or a basic amino acid residue
  VARIANT 12: note = a non-polar amino acid residue or a polar amino acid residue
  VARIANT 13: note = a peptide consisting of 2 to 6 amino acid residues
  VARIANT 14: note = a polar amino acid residue or a basic amino acid residue
GGGYIGXXXXXXXX

SEQ ID NO: 8 - protein, 14 aa, synthetic construct
  source 1..14: note = enzyme motif
  VARIANT 7: note = a peptide consisting of 6 to 12 amino acid residues
  VARIANT 8: note = a polar amino acid residue
  VARIANT 9: note = a peptide consisting of 4 to 8 amino acid residues
  VARIANT 10: note = an acidic amino acid residue or a non-polar amino acid residue
  VARIANT 11: note = a polar amino acid residue or a basic amino acid residue
  VARIANT 12: note = a non-polar amino acid residue or a polar amino acid residue
  VARIANT 13: note = a peptide consisting of 2 to 6 amino acid residues
  VARIANT 14: note = a polar amino acid residue or a basic amino acid residue
GGGYIAXXXXXXXX

SEQ ID NO: 9 - protein, 10 aa, synthetic construct
  source 1..10: note = enzyme motif
IELVEAFAES

SEQ ID NO: 10 - protein, 6 aa, synthetic construct
  source 1..6: note = enzyme motif
KQVTLV

SEQ ID NO: 11 - protein, 4 aa, synthetic construct
  source 1..4: note = enzyme motif
DRIL

SEQ ID NO: 12 - protein, 31 aa, synthetic construct
  source 1..31: note = enzyme motif
  VARIANT 2: note = a non-polar amino acid residue
  VARIANT 4: note = a non-polar amino acid residue
  VARIANT 5: note = a non-polar amino acid residue
  VARIANT 6: note = a non-polar amino acid residue
  VARIANT 17: note = a polar amino acid residue
  VARIANT 24: note = an acidic amino acid residue or a non-polar amino acid residue
  VARIANT 25: note = a polar amino acid residue or a basic amino acid residue
  VARIANT 26: note = a non-polar amino acid residue or a polar amino acid residue
  VARIANT 31: note = a polar amino acid residue or a basic amino acid residue
GXGXXXIELVEAFAESXKQVTLVXXXDRILX

SEQ ID NO: 13 - protein, 31 aa, synthetic construct
  source 1..31: note = enzyme motif
  VARIANT 6: note = a non-polar amino acid residue
  VARIANT 17: note = a polar amino acid residue
  VARIANT 24: note = an acidic amino acid residue or a non-polar amino acid residue
  VARIANT 25: note = a polar amino acid residue or a basic amino acid residue
  VARIANT 26: note = a non-polar amino acid residue or a polar amino acid residue
  VARIANT 31: note = a polar amino acid residue or a basic amino acid residue
GGGYIXIELVEAFAESXKQVTLVXXXDRILX

SEQ ID NO: 14 - protein, 31 aa, synthetic construct
  source 1..31: note = enzyme motif
  VARIANT 17: note = a polar amino acid residue
  VARIANT 24: note = an acidic amino acid residue or a non-polar amino acid residue
  VARIANT 25: note = a polar amino acid residue or a basic amino acid residue
  VARIANT 26: note = a non-polar amino acid residue or a polar amino acid residue
  VARIANT 31: note = a polar amino acid residue or a basic amino acid residue
GGGYIGIELVEAFAESXKQVTLVXXXDRILX

SEQ ID NO: 15 - protein, 31 aa, synthetic construct
  source 1..31: note = enzyme motif
  VARIANT 17: note = a polar amino acid residue
  VARIANT 24: note = an acidic amino acid residue or a non-polar amino acid residue
  VARIANT 25: note = a polar amino acid residue or a basic amino acid residue
  VARIANT 26: note = a non-polar amino acid residue or a polar amino acid residue
  VARIANT 31: note = a polar amino acid residue or a basic amino acid residue
GGGYIAIELVEAFAESXKQVTLVXXXDRILX

SEQ ID NO: 16 - protein, 451 aa, synthetic construct
  source 1..451: note = variant of SEQ ID No. 1
MKVVVVGCTHAGTAAVKTILNEHPDASVSVYERNDNVSFLSCGIALYVGGVVKDPAGLFYSSPEELASMGAKINMEHNVKNIDNENKVVVIENLKTGETFEESYDKLVMTTGSWPIIPPIDGINSENILLCKNYNQANEIIKESKNAKKIVIVGGGYIGIELVEAFAESGKQVTLVARSDRILRKYLDAEFTSVLEHDLQERGVTLALNQTVEKFVANESGAVTAVKTPVGEYEADLVILCVGFKPNTDLLKDKVEMLPNGAIVVDEYMRTSDEAIFAAGDSCAVHYNPTGGSAYIPLATNAVRMGALVGKNIVSPTVKYRGTQATSGLYLFGFNIGSTGLTENSAPHFGVEVRSVVVEDNYRPEFMPTTEKVTMKLVYEVGTNRIVGGQIMSKYDVTQSANTLSLCVQNKMTIEDLAYVDFFFQPHFDRPWNYLNILAQAAVEQERKLAK

SEQ ID NO: 17 - protein, 451 aa, synthetic construct
  source 1..451: note = variant of SEQ ID No. 1
MKVVVVGCTHAGTAAVKTILNEHPDASVSVYERNDNVSFLSCGIALYVGGVVKDPAGLFYSSPEELASMGAKINMEHNVKNIDNENKVVVIENLKTGETFEESYDKLVMTTGSWPIIPPIDGINSENILLCKNYNQANEIIKESKNAKKIVIVGGGYIAIELVEAFAESGKQVTLVARSDRILRKYLDAEFTSVLEHDLQERGVTLALNQTVEKFVANESGAVTAVKTPVGEYEADLVILCVGFKPNTDLLKDKVEMLPNGAIVVDEYMRTSDEAIFAAGDSCAVHYNPTGGSAYIPLATNAVRMGALVGKNIVSPTVKYRGTQATSGLYLFGFNIGSTGLTENSAPHFGVEVRSVVVEDNYRPEFMPTTEKVTMKLVYEVGTNRIVGGQIMSKYDVTQSANTLSLCVQNKMTIEDLAYVDFFFQPHFDRPWNYLNILAQAAVEQERKLAK

SEQ ID NO: 18 - protein, 451 aa, synthetic construct
  source 1..451: note = variant of SEQ ID No. 1
MKVVVVGCTHAGTAAVKTILNEHPDASVSVYERNDNVSFLSCGIALYVGGVVKDPAGLFYSSPEELASMGAKINMEHNVKNIDNENKVVVIENLKTGETFEESYDKLVMTTGSWPIIPPIDGINSENILLCKNYNQANEIIKESKNAKKIVIVGGGYIGIELVEAFAESNKQVTLVARSDRILRKYLDAEFTSVLEHDLQERGVTLALNQTVEKFVANESGAVTAVKTPVGEYEADLVILCVGFKPNTDLLKDKVEMLPNGAIVVDEYMRTSDEAIFAAGDSCAVHYNPTGGSAYIPLATNAVRMGALVGKNIVSPTVKYRGTQATSGLYLFGFNIGSTGLTENSAPHFGVEVRSVVVEDNYRPEFMPTTEKVTMKLVYEVGTNRIVGGQIMSKYDVTQSANTLSLCVQNKMTIEDLAYVDFFFQPHFDRPWNYLNILAQAAVEQERKLAK

SEQ ID NO: 19 - protein, 451 aa, synthetic construct
  source 1..451: note = variant of SEQ ID No. 1
MKVVVVGCTHAGTAAVKTILNEHPDASVSVYERNDNVSFLSCGIALYVGGVVKDPAGLFYSSPEELASMGAKINMEHNVKNIDNENKVVVIENLKTGETFEESYDKLVMTTGSWPIIPPIDGINSENILLCKNYNQANEIIKESKNAKKIVIVGGGYIAIELVEAFAESNKQVTLVARSDRILRKYLDAEFTSVLEHDLQERGVTLALNQTVEKFVANESGAVTAVKTPVGEYEADLVILCVGFKPNTDLLKDKVEMLPNGAIVVDEYMRTSDEAIFAAGDSCAVHYNPTGGSAYIPLATNAVRMGALVGKNIVSPTVKYRGTQATSGLYLFGFNIGSTGLTENSAPHFGVEVRSVVVEDNYRPEFMPTTEKVTMKLVYEVGTNRIVGGQIMSKYDVTQSANTLSLCVQNKMTIEDLAYVDFFFQPHFDRPWNYLNILAQAAVEQERKLAK

SEQ ID NO: 20 - DNA, 1356 bp, synthetic construct
  source 1..1356: mol_type = other DNA; note = variant of SEQ ID No.2
atgaaagtagtagtagtaggctgtacacatgcaggaacagcggcagttaagacgattttaaatgaacatccagatgcatcagtatcagtatatgagcgtaatgacaatgtctcatttctatcttgtgggattgcgttgtatgttggtggagttgtgaaagatcctgcaggtttgttttattcaagtccagaagaacttgcatcaatgggcgcgaaaattaacatggaacacaatgtgaaaaatatagataatgagaataaggtcgtagtaattgagaatttaaaaacaggcgaaacatttgaagaaagctatgataagttggtaatgacaactggatcatggccaattattcctccaattgatggaatcaatagtgaaaatattcttttgtgtaaaaactataaccaagcaaatgaaattattaaagaatcaaaaaatgctaaaaagattgtcattgttggtggtggctatattggaattgaattagttgaggcatttgcagaatctggcaagcaagtgacgctagttgcgcgtagcgatcgtattttacgtaaatatttagatgctgaattcacttctgttttagagcatgatttacaagaaagaggcgttacgctagctttaaaccaaaccgtcgagaaatttgttgccaatgaatcaggtgctgtgacagctgtgaaaacaccagttggagaatatgaggctgatttagttattttatgtgttggatttaaaccaaatactgatttgttgaaggataaagtagagatgttgccaaatggtgccatcgtagtggatgaatatatgagaacaagcgatgaagcgatttttgctgctggcgatagttgcgcggttcattataatccaactggaggctctgcgtatattccgttagctacaaatgcagttagaatgggagctttagttgggaaaaatattgtttctccaacagttaaatatcgtggcacgcaagcaacttctggtttatatttatttggttttaatataggttcaaccggattgactgaaaatagcgctcctcattttggcgtagaggttcgttcagtagttgtagaagataattatcgtccagagtttatgccgacaacagagaaagtaacgatgaaattagtttatgaagtaggaacgaatcggattgttggaggtcaaatcatgtcaaaatatgatgtgacacaatctgccaatacgttatctttatgtgttcaaaataaaatgacgattgaggatttggcttatgtagatttcttcttccaacctcactttgatcgtccttggaactatttaaatattttagcgcaagcagctgttgagcaagagcgtaaactagcaaaataa

SEQ ID NO: 21 - DNA, 1356 bp, synthetic construct
  source 1..1356: mol_type = other DNA; note = variant of SEQ ID No.2
atgaaagtagtagtagtaggctgtacacatgcaggaacagcggcagttaagacgattttaaatgaacatccagatgcatcagtatcagtatatgagcgtaatgacaatgtctcatttctatcttgtgggattgcgttgtatgttggtggagttgtgaaagatcctgcaggtttgttttattcaagtccagaagaacttgcatcaatgggcgcgaaaattaacatggaacacaatgtgaaaaatatagataatgagaataaggtcgtagtaattgagaatttaaaaacaggcgaaacatttgaagaaagctatgataagttggtaatgacaactggatcatggccaattattcctccaattgatggaatcaatagtgaaaatattcttttgtgtaaaaactataaccaagcaaatgaaattattaaagaatcaaaaaatgctaaaaagattgtcattgttggtggtggctatattgcgattgaattagttgaggcatttgcagaatctggcaagcaagtgacgctagttgcgcgtagcgatcgtattttacgtaaatatttagatgctgaattcacttctgttttagagcatgatttacaagaaagaggcgttacgctagctttaaaccaaaccgtcgagaaatttgttgccaatgaatcaggtgctgtgacagctgtgaaaacaccagttggagaatatgaggctgatttagttattttatgtgttggatttaaaccaaatactgatttgttgaaggataaagtagagatgttgccaaatggtgccatcgtagtggatgaatatatgagaacaagcgatgaagcgatttttgctgctggcgatagttgcgcggttcattataatccaactggaggctctgcgtatattccgttagctacaaatgcagttagaatgggagctttagttgggaaaaatattgtttctccaacagttaaatatcgtggcacgcaagcaacttctggtttatatttatttggttttaatataggttcaaccggattgactgaaaatagcgctcctcattttggcgtagaggttcgttcagtagttgtagaagataattatcgtccagagtttatgccgacaacagagaaagtaacgatgaaattagtttatgaagtaggaacgaatcggattgttggaggtcaaatcatgtcaaaatatgatgtgacacaatctgccaatacgttatctttatgtgttcaaaataaaatgacgattgaggatttggcttatgtagatttcttcttccaacctcactttgatcgtccttggaactatttaaatattttagcgcaagcagctgttgagcaagagcgtaaactagcaaaataa

SEQ ID NO: 22 - DNA, 1356 bp, synthetic construct
  source 1..1356: mol_type = other DNA; note = variant of SEQ ID No.2
atgaaagtagtagtagtaggctgtacacatgcaggaacagcggcagttaagacgattttaaatgaacatccagatgcatcagtatcagtatatgagcgtaatgacaatgtctcatttctatcttgtgggattgcgttgtatgttggtggagttgtgaaagatcctgcaggtttgttttattcaagtccagaagaacttgcatcaatgggcgcgaaaattaacatggaacacaatgtgaaaaatatagataatgagaataaggtcgtagtaattgagaatttaaaaacaggcgaaacatttgaagaaagctatgataagttggtaatgacaactggatcatggccaattattcctccaattgatggaatcaatagtgaaaatattcttttgtgtaaaaactataaccaagcaaatgaaattattaaagaatcaaaaaatgctaaaaagattgtcattgttggtggtggctatattggaattgaattagttgaggcatttgcagaatctaacaagcaagtgacgctagttgcgcgtagcgatcgtattttacgtaaatatttagatgctgaattcacttctgttttagagcatgatttacaagaaagaggcgttacgctagctttaaaccaaaccgtcgagaaatttgttgccaatgaatcaggtgctgtgacagctgtgaaaacaccagttggagaatatgaggctgatttagttattttatgtgttggatttaaaccaaatactgatttgttgaaggataaagtagagatgttgccaaatggtgccatcgtagtggatgaatatatgagaacaagcgatgaagcgatttttgctgctggcgatagttgcgcggttcattataatccaactggaggctctgcgtatattccgttagctacaaatgcagttagaatgggagctttagttgggaaaaatattgtttctccaacagttaaatatcgtggcacgcaagcaacttctggtttatatttatttggttttaatataggttcaaccggattgactgaaaatagcgctcctcattttggcgtagaggttcgttcagtagttgtagaagataattatcgtccagagtttatgccgacaacagagaaagtaacgatgaaattagtttatgaagtaggaacgaatcggattgttggaggtcaaatcatgtcaaaatatgatgtgacacaatctgccaatacgttatctttatgtgttcaaaataaaatgacgattgaggatttggcttatgtagatttcttcttccaacctcactttgatcgtccttggaactatttaaatattttagcgcaagcagctgttgagcaagagcgtaaactagcaaaataa

SEQ ID NO: 23 - DNA, 1356 bp, synthetic construct
  source 1..1356: mol_type = other DNA; note = variant of SEQ ID No.2
atgaaagtagtagtagtaggctgtacacatgcaggaacagcggcagttaagacgattttaaatgaacatccagatgcatcagtatcagtatatgagcgtaatgacaatgtctcatttctatcttgtgggattgcgttgtatgttggtggagttgtgaaagatcctgcaggtttgttttattcaagtccagaagaacttgcatcaatgggcgcgaaaattaacatggaacacaatgtgaaaaatatagataatgagaataaggtcgtagtaattgagaatttaaaaacaggcgaaacatttgaagaaagctatgataagttggtaatgacaactggatcatggccaattattcctccaattgatggaatcaatagtgaaaatattcttttgtgtaaaaactataaccaagcaaatgaaattattaaagaatcaaaaaatgctaaaaagattgtcattgttggtggtggctatattgcgattgaattagttgaggcatttgcagaatctaacaagcaagtgacgctagttgcgcgtagcgatcgtattttacgtaaatatttagatgctgaattcacttctgttttagagcatgatttacaagaaagaggcgttacgctagctttaaaccaaaccgtcgagaaatttgttgccaatgaatcaggtgctgtgacagctgtgaaaacaccagttggagaatatgaggctgatttagttattttatgtgttggatttaaaccaaatactgatttgttgaaggataaagtagagatgttgccaaatggtgccatcgtagtggatgaatatatgagaacaagcgatgaagcgatttttgctgctggcgatagttgcgcggttcattataatccaactggaggctctgcgtatattccgttagctacaaatgcagttagaatgggagctttagttgggaaaaatattgtttctccaacagttaaatatcgtggcacgcaagcaacttctggtttatatttatttggttttaatataggttcaaccggattgactgaaaatagcgctcctcattttggcgtagaggttcgttcagtagttgtagaagataattatcgtccagagtttatgccgacaacagagaaagtaacgatgaaattagtttatgaagtaggaacgaatcggattgttggaggtcaaatcatgtcaaaatatgatgtgacacaatctgccaatacgttatctttatgtgttcaaaataaaatgacgattgaggatttggcttatgtagatttcttcttccaacctcactttgatcgtccttggaactatttaaatattttagcgcaagcagctgttgagcaagagcgtaaactagcaaaataa